European Patent Specification EP 3 414 267 B1, published December 27, 2023. Title: Combination of Human anti-FGFR4 Antibody and Sorafenib. Applicant: Daiichi Sankyo Company, Limited Daiichi Sankyo Europe GmbH. The sequence listing filed with the application follows.

SEQUENCE LISTING (68 sequences)

SEQ ID NO: 1 - protein, 5 aa, Artificial Sequence
  U4-1-VH CDRH1
RNYMS

SEQ ID NO: 2 - protein, 5 aa, Artificial Sequence
  U4-2-VH CDRH1
KAWMS

SEQ ID NO: 3 - protein, 5 aa, Artificial Sequence
  U4-3-VH, U4-7-VH and U4-9-VH CDRH1
DYYMS

SEQ ID NO: 4 - protein, 5 aa, Artificial Sequence
  U4-4-VH and U4-8-VH CDRH1
SNYMS

SEQ ID NO: 5 - protein, 5 aa, Artificial Sequence
  U4-5-VH CDRH1
SNYMN

SEQ ID NO: 6 - protein, 5 aa, Artificial Sequence
  U4-6-VH CDRH1
DYYMN

SEQ ID NO: 7 - protein, 17 aa, Artificial Sequence
  U4-1-VH, U4-2-VH and U4-7-VH CDRH2
AISGSGGSTYYADSVKG

SEQ ID NO: 8 - protein, 17 aa, Artificial Sequence
  U4-3-VH and U4-9-VH CDRH2
TISGSGGSTYYADSVKG

SEQ ID NO: 9 - protein, 17 aa, Artificial Sequence
  U4-4-VH CDRH2
LISGSGGSTYYADSVQG

SEQ ID NO: 10 - protein, 17 aa, Artificial Sequence
  U4-5-VH CDRH2
VISYDGSNKYYADSVKG

SEQ ID NO: 11 - protein, 17 aa, Artificial Sequence
  U4-8-VH CDRH2
SISGSGGRTYYADSVKG

SEQ ID NO: 12 - protein, 17 aa, Artificial Sequence
  U4-6-VH CDRH2
AIGGSGDRTYYADSVKG

SEQ ID NO: 13 - protein, 9 aa, Artificial Sequence
  U4-1-VH CDRH3
VTSPGAFDI

SEQ ID NO: 14 - protein, 9 aa, Artificial Sequence
  U4-2-VH CDRH3
LYSYGDFDH

SEQ ID NO: 15 - protein, 9 aa, Artificial Sequence
  U4-3-VH and U4-9-VH CDRH3
LTAYGHVDS

SEQ ID NO: 16 - protein, 10 aa, Artificial Sequence
  U4-4-VH CDRH3
NTAGFGYFDL

SEQ ID NO: 17 - protein, 12 aa, Artificial Sequence
  U4-5-VH CDRH3
KSRDFWRGPFDY

SEQ ID NO: 18 - protein, 9 aa, Artificial Sequence
  U4-8-VH CDRH3
MTVFGAATL

SEQ ID NO: 19 - protein, 7 aa, Artificial Sequence
  U4-6-VH CDRH3
GGSYFGY

SEQ ID NO: 20 - protein, 9 aa, Artificial Sequence
  U4-7-VH CDRH3
LATYGPFDD

SEQ ID NO: 21 - protein, 13 aa, Artificial Sequence
  U4-1-VL CDRL1
SGGTSNIGTNTVN

SEQ ID NO: 22 - protein, 13 aa, Artificial Sequence
  U4-2-VL, U4-4-VL, U4-5-VL, U4-6-VL and U4-8-VL CDRL1
SGSSSNIGSNTVN

SEQ ID NO: 23 - protein, 13 aa, Artificial Sequence
  U4-3-VL CDRL1
SGSSSNIGTNTVN

SEQ ID NO: 24 - protein, 7 aa, Artificial Sequence
  U4-1-VL, U4-2-VL, U4-4-VL, U4-5-VL and U4-8-VL CDRL2
RNNQRPS

SEQ ID NO: 25 - protein, 7 aa, Artificial Sequence
  U4-3-VL CDRL2
RNYQRPS

SEQ ID NO: 26 - protein, 7 aa, Artificial Sequence
  U4-6-VL CDRL2
YDDLLPS

SEQ ID NO: 27 - protein, 7 aa, Artificial Sequence
  U4-7-VL and U4-9-VL CDRL2
RNNRRPS

SEQ ID NO: 28 - protein, 13 aa, Artificial Sequence
  U4-1-VL CDRL3
AAWDDSLNGPYVV

SEQ ID NO: 29 - protein, 13 aa, Artificial Sequence
  U4-2-VL CDRL3
AAWDDSLNGPAVV

SEQ ID NO: 30 - protein, 13 aa, Artificial Sequence
  U4-3-VL CDRL3
AAWDDSLSGPHVV

SEQ ID NO: 31 - protein, 13 aa, Artificial Sequence
  U4-4-VL CDRL3
AAWDDSLNGPLVV

SEQ ID NO: 32 - protein, 11 aa, Artificial Sequence
  U4-5-VL CDRL3
STWDDSLRGWV

SEQ ID NO: 33 - protein, 13 aa, Artificial Sequence
  U4-8-VL CDRL3
AAWDDSLNGPYWV

SEQ ID NO: 34 - protein, 11 aa, Artificial Sequence
  U4-6-VL CDRL3
AAWDDSLNGPV

SEQ ID NO: 35 - protein, 13 aa, Artificial Sequence
  U4-7-VL and U4-9-VL CDRL3
AAWDDSLSGPNVV

SEQ ID NO: 36 - DNA, 354 bp, Artificial Sequence
  U4-1-VH
gaggtgcagctgttggagtctgggggaggcttggtacagcctggggggtccctgagactctcctgtgcagcctctggattcaccttcagtagaaactacatgagttgggtccgccaggctccagggaaggggctggagtgggtctcagctattagtggtagtggtggtagcacatactacgcagactccgtgaagggccggttcaccatctccagagacaattccaagaacacgctgtatctgcaaatgaacagcctgagagccgaggacactgccgtgtattactgtgcgagagttacctcaccaggggcttttgatatctggggccaaggtaccctggtcaccgtgagctca

SEQ ID NO: 37 - DNA, 399 bp, Artificial Sequence
  U4-2-VH
gaggtgcagctgttggagtctgggggaggcttggtacagcctggggggtccctgagactctcctgtgcagcctctggattcaccttcagtaaagcctggatgagctgggtccgccaggctccagggaaggggctggagtgggtctcagctattagtggtagtggtggtagcacatactacgcagactccgtgaagggccggttcaccatctccagagacaattccaagaacacgctgtatctgcaaatgaacagcctgagagccgaggacactgccgtgtattactgtgcgagattatacagctatggtgactttgaccactggggccaaggtaccctggtcaccgtgagctcagcctccaccaagggcccaagcgtcttccccctggcaccctcctcc

SEQ ID NO: 38 - DNA, 399 bp, Artificial Sequence
  U4-3-VH and U4-9-VH
gaggtgcagctgttggagtctgggggaggcttggtacagcctggggggtccctgagactctcctgtgcagcctctggattcaccttcagtgactactacatgagctggatccgccaggctccagggaaggggctggagtgggtctcaactattagtggtagtggtggtagtacatactacgcagactccgtgaagggccggttcaccatctccagagacaattccaagaacacgctgtatctgcaaatgaacagcctgagagccgaggacactgccgtgtattactgtgccagactcaccgcctatggccacgtagactcctggggccaaggtaccctggtcaccgtgagctcagcctccaccaagggcccaagcgtcttccccctggcaccctcctcc

SEQ ID NO: 39 - DNA, 402 bp, Artificial Sequence
  U4-4-VH
gaggtgcagctgttggagtctgggggaggcttggtacagcctggggggtccctgagactctcctgtgcagcctctggattcaccttcagtagcaactacatgagctgggtccgccaggctccagggaaggggctggagtgggtctcacttattagtggtagtggtggtagcacatactacgcagactccgtgcagggccgcttcaccatctccagagacaattccaagaacacgctgtatctgcaaatgaacagcctgagagccgaggacactgccgtgtattactgtgcgagaaatacggctggttttgggtacttcgatctctggggccaaggtaccctggtcaccgtgagctcagcctccaccaagggcccaagcgtcttccccctggcaccctcctcc

SEQ ID NO: 40 - DNA, 408 bp, Artificial Sequence
  U4-5-VH
gaggtgcagctgttggagtctgggggaggcttggtacagcctggggggtccctgagactctcctgtgcagcctctggattcaccttcagtagcaactacatgaactgggtccgccaggctccagggaaggggctggagtgggtggcagttatatcatatgatggaagtaataaatactacgcagactccgtgaagggccgattcaccatctccagagacaattccaagaacacgctgtatctgcaaatgaacagcctgagagccgaggacactgccgtgtattactgtgtgacaaagtctcgagatttttggcggggtccctttgactactggggccaaggtaccctggtcaccgtgagctcagcctccaccaagggcccaagcgtcttccccctggcaccctcctcc

SEQ ID NO: 41 - DNA, 399 bp, Artificial Sequence
  U4-8-VH
gaggtgcagctgttggagtctgggggaggcttggtacagcctggggggtccctgagactctcctgtgcagcctctggattcaccttcagtagcaactacatgagctgggtccgccaggctccagggaaggggctggagtgggtctcaagtattagtggtagtggtggtcgcacatactacgcagactccgtgaagggccgattcaccatctccagagacaattccaagaacacgctgtatctgcaaatgaacagcctgagagccgaggacactgccgtgtattactgtgcgagaatgacggtctttggagcggcaacgctctggggccaaggtaccctggtcaccgtgagctcagcctccaccaagggcccaagcgtcttccccctggcaccctcctcc

SEQ ID NO: 42 - DNA, 393 bp, Artificial Sequence
  U4-6-VH
gaggtgcagctgttggagtctgggggaggcttggtacagcctggggggtccctgagactctcctgtgcagcctctggattcaccttcagtgactactacatgaactgggtccgccaggctccaggcaaggggctggagtgggtctcagctattggtggtagtggtgatagaacatactacgcagactccgtgaagggccggttcaccatctccagagacaattccaagaacacgctgtatctgcaaatgaacagcctgagagccgaggacactgccgtgtattactgtgctctcggtgggagctacttcggctactggggccaaggtaccctggtcaccgtgagctcagcctccaccaagggcccaagcgtcttccccctggcaccctcctcc

SEQ ID NO: 43 - DNA, 399 bp, Artificial Sequence
  U4-7-VH
gaggtgcagctgttggagtctgggggaggcttggtacagcctggggggtccctgagactctcctgtgcagcctctggattcaccttcagtgactactacatgagctgggtccgccaggctcccgggaaggggctggagtgggtctcagctattagtggtagtggtggtagcacatactacgcagactccgtgaagggccggttcaccatctccagagacaattccaagaacacgctgtatctgcaaatgaacagcctgagagccgaggacactgccgtgtattactgtgcgaccctggccacctacggaccatttgacgactggggccaaggtaccctggtcaccgtgagctcagcctccaccaagggcccaagcgtcttccccctggcaccctcctcc

SEQ ID NO: 44 - DNA, 345 bp, Artificial Sequence
  U4-1-VL
cagtctgtgctgactcagccaccctcagcgtctgggacccccgggcagagggtcaccatctcttgttctggaggcacctccaacatcggaactaatactgtaaactggtatcagcagctcccaggaacggcccccaaactcctcatctataggaataatcagcggccctcaggggtccctgaccgattctctggctccaagtctggcacctcatcctccctggccatcagtgggctccggtccgaggatgaggctgattattactgtgcagcatgggatgacagcctgaatggtccctatgtggtattcggcggaggaaccaagctgacggtcctaggtcagcct

SEQ ID NO: 45 - DNA, 345 bp, Artificial Sequence
  U4-2-VL
cagtctgtgctgactcagccaccctcagcgtctgggacccccgggcagagggtcaccatctcttgttctggaagcagctccaacatcggaagtaatactgtaaactggtatcagcagctcccaggaacggcccccaaactcctcatctatcggaataatcagcggccctcaggggtccctgaccgattctctggctccaagtctggcacctcagcctccctggccatcagtgggctccggtccgaggatgaggctgattattactgtgcagcatgggatgacagcctgaatggtcccgctgtggtattcggcggaggaaccaagctgacggtcctaggtcagcct

SEQ ID NO: 46 - DNA, 345 bp, Artificial Sequence
  U4-3-VL
cagtctgtgctgactcagccaccctcagcgtctgggacccccgggcagagggtcaccatctcttgttctggaagcagctccaacatcggaactaatactgtgaactggtatcagcagctcccaggaacggcccccaaactcctcatctataggaattatcagagaccctcaggggtccctgaccgattctctggctccaagtctggcacctcagcctccctggccatcagtgggctccggtccgaggatgaggctgattattactgtgcagcatgggatgatagcctgagtggtccacatgtggtattcggcggaggaaccaagctgacggtcctaggtcagcct

SEQ ID NO: 47 - DNA, 345 bp, Artificial Sequence
  U4-4-VL
cagtctgtgctgactcagccaccctcagcgtctgggacccccgggcagagggtcaccatctcttgttctggaagcagctccaacatcggaagtaatactgtaaactggtatcagcagctcccaggaacggcccccaaactcctcatctataggaataatcagcggccctcaggggtccctgaccgattctctggctccaagtctggcacctcagcctccctggccatcagtgggctccggtccgaggatgaggctgattattactgtgcagcatgggatgacagcctgaatggtcccctagtggtattcggcggaggaaccaagctgacggtcctaggtcagcct

SEQ ID NO: 48 - DNA, 339 bp, Artificial Sequence
  U4-5-VL
cagtctgtgctgactcagccaccctcagcgtctgggacccccgggcagagggtcaccatctcttgttctggaagcagctccaacatcggaagtaatactgtaaactggtatcagcagctcccaggaacggcccccaaactcctcatctataggaataatcagcggccctcaggggtccctgaccgattctctggctccaagtctggcacctcagcctccctggccatcagtgggctccggtccgaggatgaggctgattattactgttcaacgtgggatgacagcctgagaggttgggtgttcggcggaggaaccaagctgacggtcctaggtcagcct

SEQ ID NO: 49 - DNA, 345 bp, Artificial Sequence
  U4-8-VL
cagtctgtgctgactcagccaccctcagcatctgggacccccgggcagagggtcaccatctcttgttctggaagcagctccaacatcggaagtaatactgtaaactggtatcagcagctcccaggaacggcccccaaactcctcatctataggaataatcagcggccctcaggggtccctgaccgattctctggctccaagtctggcacctcagcctccctggccatcagtgggctccggtccgaggatgaggctgattattactgtgcagcatgggatgacagcctgaatggtccctattgggtgttcggcggaggaaccaagctgacggtcctaggtcagcct

SEQ ID NO: 50 - DNA, 339 bp, Artificial Sequence
  U4-6-VL
cagtctgtgctgactcagccaccctcagcgtctgggacccccgggcagagggtcaccatctcttgttctggaagcagctccaacatcggaagtaatactgtaaactggtatcagcagctcccaggaacggcccccaaactcctcatctattatgatgatctgctgccctcaggggtccctgaccgattctctggctccaagtctggcacctcagcctccctggccatcagtgggctccggtccgaggatgaggctgattattactgtgcagcatgggatgacagcctgaatggtccggtgttcggcggaggaaccaagctgacggtcctaggtcagcct

SEQ ID NO: 51 - DNA, 345 bp, Artificial Sequence
  U4-7-VL and U4-9-VL
cagtctgtgctgactcagccaccctcagcgtctgggacccccgggcagagggtcaccatctcttgttctggaagcagctccaacatcggaagtaatactgtacactggtatcagcagctcccaggaacggcccccaaactcctcatctatagaaataatcggcggccctcaggggtccctgaccgattctctggctccaagtctggcacctcagcctccctggccatcagtgggctccggtccgaggatgaggctgattattactgtgcagcatgggatgacagcctgagtggtccgaatgtggtattcggcggaggaaccaagctgacggtcctaggtcagcct

SEQ ID NO: 52 - protein, 118 aa, Artificial Sequence
  U4-1-VH
EVQLLESGGGLVQPGGSLRLSCAASGFTFSRNYMSWVRQAPGKGLEWVSAISGSGGSTYYADSVKGRFTISRDNSKNTLYLQMNSLRAEDTAVYYCARVTSPGAFDIWGQGTLVTVSS

SEQ ID NO: 53 - protein, 133 aa, Artificial Sequence
  U4-2-VH
EVQLLESGGGLVQPGGSLRLSCAASGFTFSKAWMSWVRQAPGKGLEWVSAISGSGGSTYYADSVKGRFTISRDNSKNTLYLQMNSLRAEDTAVYYCARLYSYGDFDHWGQGTLVTVSSASTKGPSVFPLAPSS

SEQ ID NO: 54 - protein, 133 aa, Artificial Sequence
  U4-3-VH and U4-9-VH
EVQLLESGGGLVQPGGSLRLSCAASGFTFSDYYMSWIRQAPGKGLEWVSTISGSGGSTYYADSVKGRFTISRDNSKNTLYLQMNSLRAEDTAVYYCARLTAYGHVDSWGQGTLVTVSSASTKGPSVFPLAPSS

SEQ ID NO: 55 - protein, 134 aa, Artificial Sequence
  U4-4-VH
EVQLLESGGGLVQPGGSLRLSCAASGFTFSSNYMSWVRQAPGKGLEWVSLISGSGGSTYYADSVQGRFTISRDNSKNTLYLQMNSLRAEDTAVYYCARNTAGFGYFDLWGQGTLVTVSSASTKGPSVFPLAPSS

SEQ ID NO: 56 - protein, 136 aa, Artificial Sequence
  U4-5-VH
EVQLLESGGGLVQPGGSLRLSCAASGFTFSSNYMNWVRQAPGKGLEWVAVISYDGSNKYYADSVKGRFTISRDNSKNTLYLQMNSLRAEDTAVYYCVTKSRDFWRGPFDYWGQGTLVTVSSASTKGPSVFPLAPSS

SEQ ID NO: 57 - protein, 133 aa, Artificial Sequence
  U4-8-VH
EVQLLESGGGLVQPGGSLRLSCAASGFTFSSNYMSWVRQAPGKGLEWVSSISGSGGRTYYADSVKGRFTISRDNSKNTLYLQMNSLRAEDTAVYYCARMTVFGAATLWGQGTLVTVSSASTKGPSVFPLAPSS

SEQ ID NO: 58 - protein, 131 aa, Artificial Sequence
  U4-6-VH
EVQLLESGGGLVQPGGSLRLSCAASGFTFSDYYMNWVRQAPGKGLEWVSAIGGSGDRTYYADSVKGRFTISRDNSKNTLYLQMNSLRAEDTAVYYCALGGSYFGYWGQGTLVTVSSASTKGPSVFPLAPSS

SEQ ID NO: 59 - protein, 133 aa, Artificial Sequence
  U4-7-VH
EVQLLESGGGLVQPGGSLRLSCAASGFTFSDYYMSWVRQAPGKGLEWVSAISGSGGSTYYADSVKGRFTISRDNSKNTLYLQMNSLRAEDTAVYYCATLATYGPFDDWGQGTLVTVSSASTKGPSVFPLAPSS

SEQ ID NO: 60 - protein, 115 aa, Artificial Sequence
  U4-1-VL
QSVLTQPPSASGTPGQRVTISCSGGTSNIGTNTVNWYQQLPGTAPKLLIYRNNQRPSGVPDRFSGSKSGTSSSLAISGLRSEDEADYYCAAWDDSLNGPYVVFGGGTKLTVLGQP

SEQ ID NO: 61 - protein, 115 aa, Artificial Sequence
  U4-2-VL
QSVLTQPPSASGTPGQRVTISCSGSSSNIGSNTVNWYQQLPGTAPKLLIYRNNQRPSGVPDRFSGSKSGTSASLAISGLRSEDEADYYCAAWDDSLNGPAVVFGGGTKLTVLGQP

SEQ ID NO: 62 - protein, 115 aa, Artificial Sequence
  U4-3-VL
QSVLTQPPSASGTPGQRVTISCSGSSSNIGTNTVNWYQQLPGTAPKLLIYRNYQRPSGVPDRFSGSKSGTSASLAISGLRSEDEADYYCAAWDDSLSGPHVVFGGGTKLTVLGQP

SEQ ID NO: 63 - protein, 115 aa, Artificial Sequence
  U4-4-VL
QSVLTQPPSASGTPGQRVTISCSGSSSNIGSNTVNWYQQLPGTAPKLLIYRNNQRPSGVPDRFSGSKSGTSASLAISGLRSEDEADYYCAAWDDSLNGPLVVFGGGTKLTVLGQP

SEQ ID NO: 64 - protein, 113 aa, Artificial Sequence
  U4-5-VL
QSVLTQPPSASGTPGQRVTISCSGSSSNIGSNTVNWYQQLPGTAPKLLIYRNNQRPSGVPDRFSGSKSGTSASLAISGLRSEDEADYYCSTWDDSLRGWVFGGGTKLTVLGQP

SEQ ID NO: 65 - protein, 115 aa, Artificial Sequence
  U4-8-VL
QSVLTQPPSASGTPGQRVTISCSGSSSNIGSNTVNWYQQLPGTAPKLLIYRNNQRPSGVPDRFSGSKSGTSASLAISGLRSEDEADYYCAAWDDSLNGPYWVFGGGTKLTVLGQP

SEQ ID NO: 66 - protein, 113 aa, Artificial Sequence
  U4-6-VL
QSVLTQPPSASGTPGQRVTISCSGSSSNIGSNTVNWYQQLPGTAPKLLIYYDDLLPSGVPDRFSGSKSGTSASLAISGLRSEDEADYYCAAWDDSLNGPVFGGGTKLTVLGQP

SEQ ID NO: 67 - protein, 115 aa, Artificial Sequence
  U4-7-VL and U4-9-VL
QSVLTQPPSASGTPGQRVTISCSGSSSNIGSNTVHWYQQLPGTAPKLLIYRNNRRPSGVPDRFSGSKSGTSASLAISGLRSEDEADYYCAAWDDSLSGPNVVFGGGTKLTVLGQP

SEQ ID NO: 68 - protein, 13 aa, Artificial Sequence
  U4-7 and U4-9 CDRL1
SGSSSNIGSNTVH